European Patent Application EP 4 736 867 A1, published May 6, 2026. Title: A Composition for treating spinal cord injury disorders and the Use thereof. Applicant: 주식회사 스탠드업테라퓨티스. The sequence listing filed with the application follows.

SEQUENCE LISTING (39 sequences)

SEQ ID NO: 1 - protein, 222 aa, synthetic construct
MAARPKLHYPNGRGRMESVRWVLAAAGVEFDEEFLETKEQLYKLQDGNHLLFQQVPMVEIDGMKLVQTRSILHYIADKHNLFGKNLKERTLIDMYVEGTLDLLELLIMHPFLKPDDQQKEVVNMAQKAIIRYFPVFEKILRGHGQSFLVGNQLSLADVILLQTILALEEKIPNILSAFPFLQEYTVKLSNIPTIKRFLEPGSKKKPPPDEIYVRTVYNIFRP

SEQ ID NO: 2 - DNA, 1240 bp, synthetic construct
  source 1..1240: mol_type = other DNA
gctttgtgcggctccaggcctccgagtggactccagaaagcctgaaaagctatcatggcagcaaggcccaagctccactatcccaacggaagaggccggatggagtccgtgagatgggttttagctgccgccggagtcgagtttgatgaagaatttctggaaacaaaagaacagttgtacaagttgcaggatggtaaccacctgctgttccaacaagtgcccatggttgaaattgacgggatgaagttggtacagacccgaagcattctccactacatagcagacaagcacaatctctttggcaagaacctcaaggagagaaccctgattgacatgtacgtggaggggacactggatctgctggaactgcttatcatgcatcctttcttaaaaccagatgatcagcaaaaggaagtggttaacatggcccagaaggctataattagatactttcctgtgtttgaaaagattttaaggggtcacggacaaagctttcttgttggtaatcagctgagccttgcagatgtgattttactccaaaccattttagctctagaagagaaaattcctaatatcctgtctgcatttcctttcctccaggaatacacagtgaaactaagtaatatccctacaattaagagattccttgaacctggcagcaagaagaagcctccccctgatgaaatttatgtgagaaccgtctacaacatctttaggccataaaacaacacatccatgtgtgagtgacagtgtgttcctagagatggtattgtctacagtcatgtcttaatggatcccagctctgtcatggtgctatctatgtattaagttgggtcctaagttgggtcttttgtgtcaacgagatcatctcttctagaaatatcaaccttttttgtccagtaaataattgttaggggatctttattggaaaacttttttggagaggctggtatttaagttagatctgattgggctactcatgtcctgtagccagttcatcctcataataagaatgggcaggatctcttgttctctcctgagtgtctttctactctcctgagcgtctttctgctctccttatcctgttctcttatccttatcccctccagtctctgcctaatttttagtgtttaataacaaccgaatgtctagtaaatgactctcctctgagctgtaataaataaaatggtagtaatgaatgcaatcagtattagccaaaataaagaatttatgagtcatt

SEQ ID NO: 3 - DNA, 9536 bp, synthetic construct
  source 1..9536: mol_type = other DNA
cgccatgttgacattgattattgactagttattaatagtaatcaattacggggtcattagttcatagcccatatatggagttccgcgttacataacttacggtaaatggcccgcctggctgaccgcccaacgacccccgcccattgacgtcaataatgacgtatgttcccatagtaacgccaatagggactttccattgacgtcaatgggtggagtatttacggtaaactgcccacttggcagtacatcaagtgtatcatatgccaagtacgccccctattgacgtcaatgacggtaaatggcccgcctggcattatgcccagtacatgaccttatgggactttcctacttggcagtacatctacgtattagtcatcgctattaccatggtgatgcggttttggcagtacatcaatgggcgtggatagcggtttgactcacggggatttccaagtctccaccccattgacgtcaatgggagtttgttttggcaccaaaatcaacgggactttccaaaatgtcgtaacaactccgccccattgacgcaaatgggcggtaggcgtgtacggtgggaggtctatataagcagagctcgtttagtgaaccgtcagatcgcctggagacgccatccacgctgttttgacctccatagaagacaccgggaccgatccagcctcccctcgaagcttacatgtggtaccatggaaagctctgccaagatggagagcggcggcgccggccagcagccccagccgcagccccagcagcccttcctgccgcccgcagcctgtttctttgccacggccgcagccgcggcggccgcagccgccgcagcggcagcgcagagcgcgcagcagcagcagcagcagcagcagcagcagcagcaggcgccgcagctgagaccggcggccgacggccagccctcagggggcggtcacaagtcagcgcccaagcaagtcaagcgacagcgctcgtcttcgcccgaactgatgcgctgcaaacgccggctcaacttcagcggctttggctacagcctgccgcagcagcagccggccgccgtggcgcgccgcaacgagcgcgagcgcaaccgcgtcaagttggtcaacctgggctttgccacccttcgggagcacgtccccaacggcgcggccaacaagaagatgagtaaggtggagacactgcgctcggcggtcgagtacatccgcgcgctgcagcagctgctggacgagcatgacgcggtgagcgccgccttccaggcaggcgtcctgtcgcccaccatctcccccaactactccaacgacttgaactccatggccggctcgccggtctcatcctactcgtcggacgagggctcttacgacccgctcagccccgaggagcaggagcttctcgacttcaccaactggttcggcagtggagagggcagaggaagtctgctaacatgcggtgacgtcgaggagaatcctggcccaatgttcgtcaaatccgagaccttggagttgaaggaggaagaggacgtgttagtgctgctcggatcggcctcccccgccttggcggccctgaccccgctgtcatccagcgccgacgaagaagaggaggaggagccgggcgcgtcaggcggggcgcgtcggcagcgcggggctgaggccgggcagggggcgcggggcggcgtggctgcgggtgcggagggctgccggcccgcacggctgctgggtctggtacacgattgcaaacggcgcccttcccgggcgcgggccgtctcccgaggcgccaagacggccgagacggtgcagcgcatcaagaagacccgtagactgaaggccaacaaccgcgagcgaaaccgcatgcacaacctcaacgcggcactggacgcgctgcgcgaggtgctccccacgttccccgaggacgccaagctcaccaagatcgagaccctgcgcttcgcccacaactacatctgggcactcaccgagaccctgcgcctggcggatcactgcgggggcggcggcgggggcctgccgggggcgctcttctccgaggcagtgttgctgagcccgggaggcgccagcgccgccctgagcagcagcggagacagcccctcgcccgcctccacgtggagttgcaccaacagccccgcgccgtcctcctccgtgtcctccaattccacctccccctacagctgcactttatcgcccgccagcccggccgggtcagacatggactattggcagcccccacctcccgacaagcaccgctatgcacctcacctccccatagccagggattgtatcttgggatccggagctactaacttcagcctgctgaagcaggctggagacgtggaggagaaccctggacctatgggagacatgggagatccaccaaaaaaaaaacgtctgatttccctatgtgttggttgcggcaatcagattcacgatcagtatattctgagggtttctccggatttggaatggcatgcggcatgtttgaaatgtgcggagtgtaatcagtatttggacgagagctgtacatgctttgttagggatgggaaaacctactgtaaaagagattatatcaggttgtacgggatcaaatgcgccaagtgcagcatcggcttcagcaagaacgacttcgtgatgcgtgcccgctccaaggtgtatcacatcgagtgtttccgctgtgtggcctgcagccgccagctcatccctggggacgaatttgcgcttcgggaggacggtctcttctgccgagcagaccacgatgtggtggagagggccagtctaggcgctggcgacccgctcagtcccctgcatccagcgcggccactgcaaatggcagcggagcccatctccgccaggcagccggccctgcggccccacgtccacaagcagccggagaagaccacccgcgtgcggactgtgctgaacgagaagcagctgcacaccttgcggacctgctacgccgcaaacccgcggccagatgcgctcatgaaggagcaactggtagagatgacgggcctcagtccccgtgtgatccgggtctggtttcaaaacaagcggtgcaaggacaagaagcgaagcatcatgatgaagcaactccagcagcagcagcccaatgacaaaactaatatccaggggatgacaggaactcccatggtggctgccagtccagagagacacgacggtggcttacaggctaacccagtggaagtacaaagttaccagccaccttggaaagtactgagcgacttcgccttgcagagtgacatagatcagcctgcttttcagcaactggtcaatttttcagaaggaggaccgggctctaattccactggcagtgaagtagcatcaatgtcctctcaacttccagatacacctaacagcatggtagccagtcctattgaggcattgatgcacagcagaggctctggcgagggcagaggcagcctgctgacatgtggcgacgtggaagagaaccctggccccggtaccatggaagccagaggcgaactgggccctgccagagaatctgccggcggagatctgctgctggccctgctggctagaagggccgacctgagaagagaaatccccctgtgcgccggctgcgaccagcacatcctggaccggtttatcctgaaggccctggacagacactggcacagcaagtgcctgaagtgcagcgactgccacacccccctggccgagagatgctttagcagaggcgagagcgtgtactgcaaggacgacttcttcaagagattcggcaccaagtgcgccgcctgccagctgggaattcctcctacacaggtcgtgcggagagcccaggacttcgtgtaccatctgcactgcttcgcctgcgtcgtgtgcaagagacagctggccaccggcgacgagttctacctgatggaagatagccggctcgtgtgtaaagccgactacgagacagccaagcagagagaggccgaggccaccgccaaaagacccagaaccaccatcaccgccaagcagctggaaaccctgaagtccgcctacaacaccagccccaagcccgccagacatgtgcgggaacagctgagcagcgagacaggcctggacatgagagtggtgcaagtgtggttccagaacagacgggccaaagagaagcggctgaagaaggacgccggcaggcagagatggggccagtacttccggaacatgaagcggtccagaggcggcagcaagagcgacaaggacagcgtgcaggaaggccaggacagcgacgccgaggtgtccttcccagatgagcctagcctggccgaaatgggcccagccaatggcctgtatggcagcctgggagagccaacccaggctctgggcagaccttctggcgccctgggcaacttctctctggaacacggcggactggccggacccgagcagtatagagaactgaggcccggcagcccttacggcgtgccaccttctccagctgcccctcagtctctgccaggacctcagcctctgctgtccagcctggtgtaccccgatacaagcctgggcctggtgccatctggcgctccaggcggacctcctccaatgagagtgctggccggcaatggccctagcagcgatctgagcacaggcagctctggcggctaccccgattttcctgccagccctgcctcctggctggacgaagtggatcacgcccagttctgagcggccgctctagaggatccaagcttatcgataccgtcgacctcgagggcccagatctaattcaccccaccagtgcaggctgcctatcagaaagtggtggctggtgtggctaatgccctggcccacaagtatcactaagctcgctttcttgctgtccaatttctattaaaggttcctttgttccctaagtccaactactaaactgggggatattatgaagggccttgagcatctggattctgcctaataaaaaacatttattttcattgcaatgatgtatttaaattatttctgaatattttactaaaaagggaatgtgggaggtcagtgcatttaaaacataaagaaatgaagagctagttcaaaccttgggaaaatacactatatcttaaactccatgaaagaaggtgaggctgcaaacagctaatgcacattggcaacagcccctgatgcctatgccttattcatccctcagaaaaggattcaagtagaggcttgatttggaggttaaagttttgctatgctgtattttacattacttattgttttagctgtcctcatgaatgtcttttcactacccatttgcttatcctgcatctctcagccttgactccactcagttctcttgcttagagataccacctttcccctgaagtgttccttccatgttttacggcgagatggtttctcctcgcctggccactcagccttagttgtctctgttgtcttatagaggtctacttgaagaaggaaaaacagggggcatggtttgactgtcctgtgagcccttcttccctgcctcccccactcacagtgacccggaatccctcgacatctagagcatggctacgtagataagtagcatggcgggttaatcattaactacaaggaacccctagtgatggagttggccactccctctctgcgcgctcgctcgctcactgaggccgggcgaccaaaggtcgcccgacgcccgggctttgcccgggcggcctcagtgagcgagcgagcgcgcagctggcgtaatagcgaagaggcccgcaccgatcgcccttcccaacagttgcgcagcctgaatggcgaatggcgattccgttgcaatggctggcggtaatattgttctggatattaccagcaaggccgatagtttgagttcttctactcaggcaagtgatgttattactaatcaaagaagtattgcgacaacggttaatttgcgtgatggacagactcttttactcggtggcctcactgattataaaaacacttctcaggattctggcgtaccgttcctgtctaaaatccctttaatcggcctcctgtttagctcccgctctgattctaacgaggaaagcacgttatacgtgctcgtcaaagcaaccatagtacgcgccctgtagcggcgcattaagcgcggcgggtgtggtggttacgcgcagcgtgaccgctacacttgccagcgccctagcgcccgctcctttcgctttcttcccttcctttctcgccacgttcgccggctttccccgtcaagctctaaatcgggggctccctttagggttccgatttagtgctttacggcacctcgaccccaaaaaacttgattagggtgatggttcacgtagtgggccatcgccctgatagacggtttttcgccctttgacgttggagtccacgttctttaatagtggactcttgttccaaactggaacaacactcaaccctatctcggtctattcttttgatttataagggattttgccgatttcggcctattggttaaaaaatgagctgatttaacaaaaatttaacgcgaattttaacaaaatattaacgcttacaatttaaatatttgcttatacaatcttcctgtttttggggcttttctgattatcaaccggggtacatatgattgacatgctagttttacgattaccgttcatcgattctcttgtttgctccagactctcaggcaatgacctgatagcctttgtagagacctctcaaaaatagctaccctctccggcatgaatttatcagctagaacggttgaatatcatattgatggtgatttgactgtctccggcctttctcacccgtttgaatctttacctacacattactcaggcattgcatttaaaatatatgagggttctaaaaatttttatccttgcgttgaaataaaggcttctcccgcaaaagtattacagggtcataatgtttttggtacaaccgatttagctttatgctctgaggctttattgcttaattttgctaattctttgccttgcctgtatgatttattggatgttggaatcgcctgatgcggtattttctccttacgcatctgtgcggtatttcacaccgcatatggtgcactctcagtacaatctgctctgatgccgcatagttaagccagccccgacacccgccaacacccgctgacgcgccctgacgggcttgtctgctcccggcatccgcttacagacaagctgtgaccgtctccgggagctgcatgtgtcagaggttttcaccgtcatcaccgaaacgcgcgagacgaaagggcctcgtgatacgcctatttttataggttaatgtcatgataataatggtttcttagacgtcaggtggcacttttcggggaaatgtgcgcggaacccctatttgtttatttttctaaatacattcaaatatgtatccgctcatgagacaataaccctgataaatgcttcaataatattgaaaaaggaagagtatgattgaacaagatggattgcacgcaggttctccggccgcttgggtggagaggctattcggctatgactgggcacaacagacaatcggctgctctgatgccgccgtgttccggctgtcagcgcaggggcgcccggttctttttgtcaagaccgacctgtccggtgccctgaatgaactgcaagacgaggcagcgcggctatcgtggctggccacgacgggcgttccttgcgcagctgtgctcgacgttgtcactgaagcgggaagggactggctgctattgggcgaagtgccggggcaggatctcctgtcatctcaccttgctcctgccgagaaagtatccatcatggctgatgcaatgcggcggctgcatacgcttgatccggctacctgcccattcgaccaccaagcgaaacatcgcatcgagcgagcacgtactcggatggaagccggtcttgtcgatcaggatgatctggacgaagagcatcaggggctcgcgccagccgaactgttcgccaggctcaaggcgagcatgcccgacggcgaggatctcgtcgtgacccatggcgatgcctgcttgccgaatatcatggtggaaaatggccgcttttctggattcatcgactgtggccggctgggtgtggcggaccgctatcaggacatagcgttggctacccgtgatattgctgaagagcttggcggcgaatgggctgaccgcttcctcgtgctttacggtatcgccgctcccgattcgcagcgcatcgccttctatcgccttcttgacgagttcttctgactgtcagaccaagtttactcatatatactttagattgatttaaaacttcatttttaatttaaaaggatctaggtgaagatcctttttgataatctcatgaccaaaatcccttaacgtgagttttcgttccactgagcgtcagaccccgtagaaaagatcaaaggatcttcttgagatcctttttttctgcgcgtaatctgctgcttgcaaacaaaaaaaccaccgctaccagcggtggtttgtttgccggatcaagagctaccaactctttttccgaaggtaactggcttcagcagagcgcagataccaaatactgttcttctagtgtagccgtagttaggccaccacttcaagaactctgtagcaccgcctacatacctcgctctgctaatcctgttaccagtggctgctgccagtggcgataagtcgtgtcttaccgggttggactcaagacgatagttaccggataaggcgcagcggtcgggctgaacggggggttcgtgcacacagcccagcttggagcgaacgacctacaccgaactgagatacctacagcgtgagctatgagaaagcgccacgcttcccgaagggagaaaggcggacaggtatccggtaagcggcagggtcggaacaggagagcgcacgagggagcttccagggggaaacgcctggtatctttatagtcctgtcgggtttcgccacctctgacttgagcgtcgatttttgtgatgctcgtcaggggggcggagcctatggaaaaacgccagcaacgcggcctttttacggttcctggccttttgctggccttttgctcacatgttctttcctgcgttatcccctgattctgtggataaccgtattaccgcctttgagtgagctgataccgctcgccgcagccgaacgaccgagcgcagcgagtcagtgagcgaggaagcggaagagcgcccaatacgcaaaccgcctctccccgcgcgttggccgattcattaatgcagctgcgcgctcgctcgctcactgaggccgcccgggcaaagcccgggcgtcgggcgacctttggtcgcccggcctcagtgagcgagcgagcgcgcagagagggagtggccaactccatcactaggggttccttgtagttaatgattaacccgccatgctacttatctacgtagccatgctctagcggcctcggcctctgcataaataaaaaaaattagtcagccatgagcttggcccattgcatacgttgtatccatatcataatatgtacatttatattggctcatgtccaacattac

SEQ ID NO: 4 - DNA, 9271 bp, synthetic construct
  source 1..9271: mol_type = other DNA
cgccatgttgacattgattattgactagttattaatagtaatcaattacggggtcattagttcatagcccatatatggagttccgcgttacataacttacggtaaatggcccgcctggctgaccgcccaacgacccccgcccattgacgtcaataatgacgtatgttcccatagtaacgccaatagggactttccattgacgtcaatgggtggagtatttacggtaaactgcccacttggcagtacatcaagtgtatcatatgccaagtacgccccctattgacgtcaatgacggtaaatggcccgcctggcattatgcccagtacatgaccttatgggactttcctacttggcagtacatctacgtattagtcatcgctattaccatggtgatgcggttttggcagtacatcaatgggcgtggatagcggtttgactcacggggatttccaagtctccaccccattgacgtcaatgggagtttgttttggcaccaaaatcaacgggactttccaaaatgtcgtaacaactccgccccattgacgcaaatgggcggtaggcgtgtacggtgggaggtctatataagcagagctcgtttagtgaaccgtcagatcgcctggagacgccatccacgctgttttgacctccatagaagacaccgggaccgatccagcctcccctcgaagcttacatgtggtaccatggcgaccgcagcgtctaaccactacagcctgctcacctccagcgcctccatcgtgcacgccgagccgcccggcggcatgcagcagggcgcggggggctaccgcgaagcgcagagcctggtgcagggcgactacggcgctctgcagagcaacggacacccgctcagccacgctcaccagtggatcaccgcgctgtcccacggcggcggcggcgggggcggtggcggcggcggggggggcgggggcggcggcgggggcggcggcgacggctccccgtggtccaccagccccctgggccagccggacatcaagccctcggtggtggtgcagcagggcggccgcggagacgagctgcacgggccaggcgccctgcagcagcagcatcagcagcagcaacagcaacagcagcagcaacagcagcaacagcagcagcagcagcagcaacagcggccgccgcatctggtgcaccacgccgctaaccaccacccgggacccggggcatggcggagcgcggcggctgcagcgcacctcccaccctccatgggagcgtccaacggcggcttgctctactcgcagcccagcttcacggtgaacggcatgctgggcgccggcgggcagccggccgggctgcaccaccacggcctgcgggacgcgcacgacgagccacaccatgccgaccaccacccgcacccgcactcgcacccacaccagcagccgccgcccccgccgcccccgcagggtccgcctggccacccaggcgcgcaccacgacccgcactcggacgaggacacgccgacctcggacgacctggagcagttcgccaagcagttcaagcagcggcggatcaaactgggatttacccaagcggacgtggggctggctctgggcaccctgtatggcaacgtgttctcgcagaccaccatctgcaggtttgaggccctgcagctgagcttcaagaacatgtgcaagctgaagcctttgttgaacaagtggttggaggaggcggactcgtcctcgggcagccccacgagcatagacaagatcgcagcgcaagggcgcaagcggaaaaagcggacctccatcgaggtgagcgtcaagggggctctggagagccatttcctcaaatgccccaagccctcggcccaggagatcacctccctcgcggacagcttacagctggagaaggaggtggtgagagtttggttttgtaacaggagacagaaagagaaaaggatgacccctcccggagggactctgccgggcgccgaggatgtgtacggggggagtagggacactccaccacaccacggggtgcagacgcccgtccagggtagcggtgccactaacttctccctgttgaaacaagcaggggatgtcgaagagaatcctggtccaatggaaaaatccaaaaatttccgcatcgacgccctgctggcggtggaccccccacgagccgcctctgcgcagagcgcgccgctggccttggtcacgtcgctcgccgccgccgcatctggcaccggaggtggcggcggcggcggcggggcgagcggcgggactagcggcagctgcagccccgcgtcctcggagccgccggctgcgcccgccgaccgcctgcgcgccgagagcccgtcgccgccgcgcctgctggccgcgcactgcgcgctgctgcccaagccgggcttcctgggcgcgggcggcggcggcggcggcacgggcggcgggcacggggggccccaccaccacgcgcatccgggcgcagcggccgctgccgccgccgccgccgccgccgccgccgctgggggcctggcgctggggctgcaccctgggggcgcgcagggcggcgcgggcctcccggcgcaggcggcgctctacggccacccggtctacggctactccgcggcggcggcggcggctgcgctggcgggccagcacccggcgctctcctactcgtacccgcaggtgcaaggcgcgcaccccgcgcaccccgccgaccccatcaagctgggcgccggcaccttccagctggaccagtggctgcgcgcgtccaccgcgggcatgatcctgcctaagatgcccgacttcaactcccaggcgcagtcgaacctcctggggaagtgccgccggccgcgcaccgccttcaccagccagcagctgctggagctggagcaccagttcaagctcaacaagtacctgtcgcggcccaagcgcttcgaggtggccacctcgctcatgctcaccgagacccaggtgaagatttggttccagaaccggcggatgaaatggaaacgcagcaaaaaggccaaagagcaggcggcgcaggaagcggagaaacagaagggcggcggcgggggcgcggggaagggcggcgcggaggagccgggagccgaggagctgctggggccgccagcgcccggagacaagggcagcggacgccgcctgcgggacttgagggacagtgaccccgaggaggacgaggacgaggacgacgaggaccatttcccctacagcaacggcgccagcgtccacgccgcctcctccgactgctcctcggaggacgactcgccgcccccgcggcccagccaccagcccgcgccccagggcagtggagagggcagaggaagtctgctaacatgcggtgacgtcgaggagaatcctggcccaatgaccaaatcgtacagcgagagtgggctgatgggcgagcctcagccccaaggtcctccaagctggacagacgagtgtctcagttctcaggacgaggagcacgaggcagacaagaaggaggacgacctcgaagccatgaacgcagaggaggactcactgaggaacgggggagaggaggaggacgaagatgaggacctggaagaggaggaagaagaggaagaggaggatgacgatcaaaagcccaagagacgcggccccaaaaagaagaagatgactaaggctcgcctggagcgttttaaattgagacgcatgaaggctaacgcccgggagcggaaccgcatgcacggactgaacgcggcgctagacaacctgcgcaaggtggtgccttgctattctaagacgcagaagctgtccaaaatcgagactctgcgcttggccaagaactacatctgggctctgtcggagatcctgcgctcaggcaaaagcccagacctggtctccttcgttcagacgctttgcaagggcttatcccaacccaccaccaacctggttgcgggctgcctgcaactcaatcctcggacttttctgcctgagcagaaccaggacatgcccccccacctgccgacggccagcgcttccttccctgtacacccctactcctaccagtcgcctgggctgcccagtccgccttacggtaccatggacagctcccatgtcttccacgttaagcctccgccgcacgcctacagcgcagcgctggagcccttctttgaaagccctctgactgattgcaccagcccttcctttgatggacccctcagcccgccgctcagcatcaatggcaacttctctttcaaacacgaaccgtccgccgagtttgagaaaaattatgcctttaccatgcactatcctgcagcgacactggcaggggcccaaagccacggatcaatcttctcaggcaccgctgcccctcgctgcgagatccccatagacaatattatgtccttcgatagccattcacatcatgagcgagtcatgagtgcccagctcaatgccatatttcatgattagcggccgctctagaggatccaagcttatcgataccgtcgacctcgagggcccagatctaattcaccccaccagtgcaggctgcctatcagaaagtggtggctggtgtggctaatgccctggcccacaagtatcactaagctcgctttcttgctgtccaatttctattaaaggttcctttgttccctaagtccaactactaaactgggggatattatgaagggccttgagcatctggattctgcctaataaaaaacatttattttcattgcaatgatgtatttaaattatttctgaatattttactaaaaagggaatgtgggaggtcagtgcatttaaaacataaagaaatgaagagctagttcaaaccttgggaaaatacactatatcttaaactccatgaaagaaggtgaggctgcaaacagctaatgcacattggcaacagcccctgatgcctatgccttattcatccctcagaaaaggattcaagtagaggcttgatttggaggttaaagttttgctatgctgtattttacattacttattgttttagctgtcctcatgaatgtcttttcactacccatttgcttatcctgcatctctcagccttgactccactcagttctcttgcttagagataccacctttcccctgaagtgttccttccatgttttacggcgagatggtttctcctcgcctggccactcagccttagttgtctctgttgtcttatagaggtctacttgaagaaggaaaaacagggggcatggtttgactgtcctgtgagcccttcttccctgcctcccccactcacagtgacccggaatccctcgacatctagagcatggctacgtagataagtagcatggcgggttaatcattaactacaaggaacccctagtgatggagttggccactccctctctgcgcgctcgctcgctcactgaggccgggcgaccaaaggtcgcccgacgcccgggctttgcccgggcggcctcagtgagcgagcgagcgcgcagctggcgtaatagcgaagaggcccgcaccgatcgcccttcccaacagttgcgcagcctgaatggcgaatggcgattccgttgcaatggctggcggtaatattgttctggatattaccagcaaggccgatagtttgagttcttctactcaggcaagtgatgttattactaatcaaagaagtattgcgacaacggttaatttgcgtgatggacagactcttttactcggtggcctcactgattataaaaacacttctcaggattctggcgtaccgttcctgtctaaaatccctttaatcggcctcctgtttagctcccgctctgattctaacgaggaaagcacgttatacgtgctcgtcaaagcaaccatagtacgcgccctgtagcggcgcattaagcgcggcgggtgtggtggttacgcgcagcgtgaccgctacacttgccagcgccctagcgcccgctcctttcgctttcttcccttcctttctcgccacgttcgccggctttccccgtcaagctctaaatcgggggctccctttagggttccgatttagtgctttacggcacctcgaccccaaaaaacttgattagggtgatggttcacgtagtgggccatcgccctgatagacggtttttcgccctttgacgttggagtccacgttctttaatagtggactcttgttccaaactggaacaacactcaaccctatctcggtctattcttttgatttataagggattttgccgatttcggcctattggttaaaaaatgagctgatttaacaaaaatttaacgcgaattttaacaaaatattaacgcttacaatttaaatatttgcttatacaatcttcctgtttttggggcttttctgattatcaaccggggtacatatgattgacatgctagttttacgattaccgttcatcgattctcttgtttgctccagactctcaggcaatgacctgatagcctttgtagagacctctcaaaaatagctaccctctccggcatgaatttatcagctagaacggttgaatatcatattgatggtgatttgactgtctccggcctttctcacccgtttgaatctttacctacacattactcaggcattgcatttaaaatatatgagggttctaaaaatttttatccttgcgttgaaataaaggcttctcccgcaaaagtattacagggtcataatgtttttggtacaaccgatttagctttatgctctgaggctttattgcttaattttgctaattctttgccttgcctgtatgatttattggatgttggaatcgcctgatgcggtattttctccttacgcatctgtgcggtatttcacaccgcatatggtgcactctcagtacaatctgctctgatgccgcatagttaagccagccccgacacccgccaacacccgctgacgcgccctgacgggcttgtctgctcccggcatccgcttacagacaagctgtgaccgtctccgggagctgcatgtgtcagaggttttcaccgtcatcaccgaaacgcgcgagacgaaagggcctcgtgatacgcctatttttataggttaatgtcatgataataatggtttcttagacgtcaggtggcacttttcggggaaatgtgcgcggaacccctatttgtttatttttctaaatacattcaaatatgtatccgctcatgagacaataaccctgataaatgcttcaataatattgaaaaaggaagagtatgattgaacaagatggattgcacgcaggttctccggccgcttgggtggagaggctattcggctatgactgggcacaacagacaatcggctgctctgatgccgccgtgttccggctgtcagcgcaggggcgcccggttctttttgtcaagaccgacctgtccggtgccctgaatgaactgcaagacgaggcagcgcggctatcgtggctggccacgacgggcgttccttgcgcagctgtgctcgacgttgtcactgaagcgggaagggactggctgctattgggcgaagtgccggggcaggatctcctgtcatctcaccttgctcctgccgagaaagtatccatcatggctgatgcaatgcggcggctgcatacgcttgatccggctacctgcccattcgaccaccaagcgaaacatcgcatcgagcgagcacgtactcggatggaagccggtcttgtcgatcaggatgatctggacgaagagcatcaggggctcgcgccagccgaactgttcgccaggctcaaggcgagcatgcccgacggcgaggatctcgtcgtgacccatggcgatgcctgcttgccgaatatcatggtggaaaatggccgcttttctggattcatcgactgtggccggctgggtgtggcggaccgctatcaggacatagcgttggctacccgtgatattgctgaagagcttggcggcgaatgggctgaccgcttcctcgtgctttacggtatcgccgctcccgattcgcagcgcatcgccttctatcgccttcttgacgagttcttctgactgtcagaccaagtttactcatatatactttagattgatttaaaacttcatttttaatttaaaaggatctaggtgaagatcctttttgataatctcatgaccaaaatcccttaacgtgagttttcgttccactgagcgtcagaccccgtagaaaagatcaaaggatcttcttgagatcctttttttctgcgcgtaatctgctgcttgcaaacaaaaaaaccaccgctaccagcggtggtttgtttgccggatcaagagctaccaactctttttccgaaggtaactggcttcagcagagcgcagataccaaatactgttcttctagtgtagccgtagttaggccaccacttcaagaactctgtagcaccgcctacatacctcgctctgctaatcctgttaccagtggctgctgccagtggcgataagtcgtgtcttaccgggttggactcaagacgatagttaccggataaggcgcagcggtcgggctgaacggggggttcgtgcacacagcccagcttggagcgaacgacctacaccgaactgagatacctacagcgtgagctatgagaaagcgccacgcttcccgaagggagaaaggcggacaggtatccggtaagcggcagggtcggaacaggagagcgcacgagggagcttccagggggaaacgcctggtatctttatagtcctgtcgggtttcgccacctctgacttgagcgtcgatttttgtgatgctcgtcaggggggcggagcctatggaaaaacgccagcaacgcggcctttttacggttcctggccttttgctggccttttgctcacatgttctttcctgcgttatcccctgattctgtggataaccgtattaccgcctttgagtgagctgataccgctcgccgcagccgaacgaccgagcgcagcgagtcagtgagcgaggaagcggaagagcgcccaatacgcaaaccgcctctccccgcgcgttggccgattcattaatgcagctgcgcgctcgctcgctcactgaggccgcccgggcaaagcccgggcgtcgggcgacctttggtcgcccggcctcagtgagcgagcgagcgcgcagagagggagtggccaactccatcactaggggttccttgtagttaatgattaacccgccatgctacttatctacgtagccatgctctagcggcctcggcctctgcataaataaaaaaaattagtcagccatgagcttggcccattgcatacgttgtatccatatcataatatgtacatttatattggctcatgtccaacattac

SEQ ID NO: 5 - DNA, 9827 bp, synthetic construct
  source 1..9827: mol_type = other DNA
cgccatgttgacattgattattgactagttattaatagtaatcaattacggggtcattagttcatagcccatatatggagttccgcgttacataacttacggtaaatggcccgcctggctgaccgcccaacgacccccgcccattgacgtcaataatgacgtatgttcccatagtaacgccaatagggactttccattgacgtcaatgggtggagtatttacggtaaactgcccacttggcagtacatcaagtgtatcatatgccaagtacgccccctattgacgtcaatgacggtaaatggcccgcctggcattatgcccagtacatgaccttatgggactttcctacttggcagtacatctacgtattagtcatcgctattaccatggtgatgcggttttggcagtacatcaatgggcgtggatagcggtttgactcacggggatttccaagtctccaccccattgacgtcaatgggagtttgttttggcaccaaaatcaacgggactttccaaaatgtcgtaacaactccgccccattgacgcaaatgggcggtaggcgtgtacggtgggaggtctatataagcagagctcgtttagtgaaccgtcagatcgcctggagacgccatccacgctgttttgacctccatagaagacaccgggaccgatccagcctcccctcgaagcttacatgtggtaccatggcagcaaggcccaagctccactatcccaacggaagaggccggatggagtccgtgagatgggttttagctgccgccggagtcgagtttgatgaagaatttctggaaacaaaagaacagttgtacaagttgcaggatggtaaccacctgctgttccaacaagtgcccatggttgaaattgacgggatgaagttggtacagacccgaagcattctccactacatagcagacaagcacaatctctttggcaagaacctcaaggagagaaccctgattgacatgtacgtggaggggacactggatctgctggaactgcttatcatgcatcctttcttaaaaccagatgatcagcaaaaggaagtggttaacatggcccagaaggctataattagatactttcctgtgtttgaaaagattttaaggggtcacggacaaagctttcttgttggtaatcagctgagccttgcagatgtgattttactccaaaccattttagctctagaagagaaaattcctaatatcctgtctgcatttcctttcctccaggaatacacagtgaaactaagtaatatccctacaattaagagattccttgaacctggcagcaagaagaagcctccccctgatgaaatttatgtgagaaccgtctacaacatctttaggccaggtagcggtgccactaacttctccctgttgaaacaagcaggggatgtcgaagagaatcctggtccaatggaggtggacaccgaggagaagcggcatcgcacgcggtccaaaggggttcgagttcccgtggaaccagccatacaagagctgttcagctgtcccacccctggctgtgacggcagtggtcatgtcagtggcaaatatgcaagacacagaagtgtatatggttgtcccttggcgaaaaaaagaaaaacacaagataaacagccccaggaacctgctcctaaacgaaagccatttgccgtgaaagcagacagctcctcagtggatgagtgtgacgacagtgatgggactgaggacatggatgagaaggaggaggatgagggggaggagtactccgaggacaatgacgagccaggggatgaggacgaggaggacgaggagggggaccgggaggaggaggaggagatcgaggaggaggatgaggacgatgacgaggatggagaagatgtggaggatgaagaagaggaagaggaggaggaggaggaggaggaagaggaagaagaaaacgaagaccatcaaatgaattgtcacaatactcgaataatgcaagacacagaaaaggatgataacaataatgacgaatatgacaattacgatgaactggtggccaagtcattgttaaacctcggcaaaatcgctgaggatgcagcctaccgggccaggactgagtcagaaatgaacagcaatacctccaatagtctggaagacgatagtgacaaaaacgaaaacctgggtcggaaaagtgagttgagtttagacttagacagtgatgttgttagagaaacagtggactcccttaaactattagcccaaggacacggtgttgtgctctcagaaaacatgaatgacagaaattatgcagacagcatgtcgcagcaagacagtagaaatatgaattacgtcatgttggggaagcccatgaacaatggactcatggaaaagatggtggaggagagcgatgaggaggtgtgtctgagcagtctggagtgtttgaggaatcagtgcttcgacctggccaggaagctcagtgagaccaacccgcaggagaggaatccgcagcagaacatgaacatccgtcagcatgtccggccagaagaggacttcccaggaaggacgccggacagaaactactcggacatgctgaacctcatgcggctggaggagcagttgagcccccggtcgagagtgtttgccagctgtgcgaaggaggatgggtgtcatgagcgggacgacgataccacctctgtgaactcggacaggtctgaagaggtgttcgacatgaccaaggggaacctgaccctgctggagaaagccatcgctttggaaacggaaagagcaaaggccatgagggagaagatggccatggaagctgggaggagggacaatatgaggtcatatgaggaccagtctccgagacaacttcccggggaggacagaaagcctaaatccagtgacagccatgtcaaaaagccatactatgatccctcaagaacagaaaagaaagagagcaagtgtccaacccccgggtgtgatggaaccggccacgtaactgggctgtacccacatcaccgcagcctgtccggatgcccgcacaaagatagggtccctccagaaatccttgccatgcatgaaagtgtcctcaagtgccccactccgggctgcacggggcgcgggcatgtcaacagcaacaggaactcccaccgaagcctctccggatgcccgatcgctgcagcagagaaactggccaaggcacaggaaaagcaccagagctgcgacgtgtccaagtccagccaggcctcggaccgcgtgctcaggccaatgtgctttgtgaagcagctggagattcctcagtatggctacagaaacaatgtccccacaactacgccgcgttccaacctggccaaggagctcgagaaatattccaagacctcgtttgaatacaacagttacgacaaccatacttatggcaagcgagccatagctcccaaggtgcaaaccagggatatatcccccaaaggatatgatgatgcgaagcggtactgcaaggaccccagccccagcagcagcagcaccagcagctacgcgcccagcagcagcagcaacctgagctgcggcgggggcagcagcgccagcagcacgtgcagcaagagcagcttcgactacacgcacgacatggaggcggcccacatggcggccaccgccatcctcaacctgtccacgcgctgccgcgagatgccgcagaacctgagcaccaagccgcaggacctgtgcgccacgcggaaccctgacatggaggtggatgagaacgggaccctggacctcagcatgaacaagcagaggccgcgggacagctgctgccccatcctgacccctctggagcccatgtccccccagcagcaggcagtgatgaacaaccggtgtttccagctgggcgagggcgactgctgggacttgcccgtagactacaccaaaatgaaaccccggaggatagacgaggacgagtccaaagacattactccagaagacttggacccattccaggaggctctagaagaaagacggtatcccggggaggtgaccatcccaagtcccaaacccaagtaccctcagtgcaaggagagcaaaaaggacttaataactctgtctggctgccccctggcggacaaaagcattcgaagtatgctggccaccagctcccaagaactcaagtgccccacgcctggctgtgatggttctggacatatcaccggcaattatgcttctcatcggagcctttcaggttgcccaagagcaaagaaaagtggtatcaggatagcacagagcaaagaagataaagaagatcaagaacccatcaggtgtccggtccccgggtgcgacggccagggccacatcactgggaagtacgcgtcccatcgcagcgcctccgggtgccccttggcggccaagaggcagaaagacgggtacctgaatggctcccagttctcctggaagtcggtcaagacggaaggcatgtcctgccccacgccaggatgcgacggctcaggccacgtcagcggcagcttcctcacacaccgcagcttgtcaggatgcccgagagccacgtcagcgatgaagaaggcaaagctttctggagagcagatgctgaccatcaaacagcgggccagcaacggtatagaaaatgatgaagaaatcaaacagttagatgaagaaatcaaggagctaaatgaatccaattcccagatggaagccgatatgattaaactcagaactcagattaccacgatggagagcaacctgaagaccatcgaagaggagaacaaagtgattgagcagcagaacgagtctctcctccacgagctggcgaacctgagccagtctctgatccacagcctggctaacatccagctgccgcacatggatccaatcaatgaacaaaattttgatgcttacgtgactactttgacggaaatgtatacaaatcaagatcgttatcagagtccagaaaataaagccctactggaaaatataaagcaggctgtgagaggaattcaggtctgagcggccgctctagaggatccaagcttatcgataccgtcgacctcgagggcccagatctaattcaccccaccagtgcaggctgcctatcagaaagtggtggctggtgtggctaatgccctggcccacaagtatcactaagctcgctttcttgctgtccaatttctattaaaggttcctttgttccctaagtccaactactaaactgggggatattatgaagggccttgagcatctggattctgcctaataaaaaacatttattttcattgcaatgatgtatttaaattatttctgaatattttactaaaaagggaatgtgggaggtcagtgcatttaaaacataaagaaatgaagagctagttcaaaccttgggaaaatacactatatcttaaactccatgaaagaaggtgaggctgcaaacagctaatgcacattggcaacagcccctgatgcctatgccttattcatccctcagaaaaggattcaagtagaggcttgatttggaggttaaagttttgctatgctgtattttacattacttattgttttagctgtcctcatgaatgtcttttcactacccatttgcttatcctgcatctctcagccttgactccactcagttctcttgcttagagataccacctttcccctgaagtgttccttccatgttttacggcgagatggtttctcctcgcctggccactcagccttagttgtctctgttgtcttatagaggtctacttgaagaaggaaaaacagggggcatggtttgactgtcctgtgagcccttcttccctgcctcccccactcacagtgacccggaatccctcgacatctagagcatggctacgtagataagtagcatggcgggttaatcattaactacaaggaacccctagtgatggagttggccactccctctctgcgcgctcgctcgctcactgaggccgggcgaccaaaggtcgcccgacgcccgggctttgcccgggcggcctcagtgagcgagcgagcgcgcagctggcgtaatagcgaagaggcccgcaccgatcgcccttcccaacagttgcgcagcctgaatggcgaatggcgattccgttgcaatggctggcggtaatattgttctggatattaccagcaaggccgatagtttgagttcttctactcaggcaagtgatgttattactaatcaaagaagtattgcgacaacggttaatttgcgtgatggacagactcttttactcggtggcctcactgattataaaaacacttctcaggattctggcgtaccgttcctgtctaaaatccctttaatcggcctcctgtttagctcccgctctgattctaacgaggaaagcacgttatacgtgctcgtcaaagcaaccatagtacgcgccctgtagcggcgcattaagcgcggcgggtgtggtggttacgcgcagcgtgaccgctacacttgccagcgccctagcgcccgctcctttcgctttcttcccttcctttctcgccacgttcgccggctttccccgtcaagctctaaatcgggggctccctttagggttccgatttagtgctttacggcacctcgaccccaaaaaacttgattagggtgatggttcacgtagtgggccatcgccctgatagacggtttttcgccctttgacgttggagtccacgttctttaatagtggactcttgttccaaactggaacaacactcaaccctatctcggtctattcttttgatttataagggattttgccgatttcggcctattggttaaaaaatgagctgatttaacaaaaatttaacgcgaattttaacaaaatattaacgcttacaatttaaatatttgcttatacaatcttcctgtttttggggcttttctgattatcaaccggggtacatatgattgacatgctagttttacgattaccgttcatcgattctcttgtttgctccagactctcaggcaatgacctgatagcctttgtagagacctctcaaaaatagctaccctctccggcatgaatttatcagctagaacggttgaatatcatattgatggtgatttgactgtctccggcctttctcacccgtttgaatctttacctacacattactcaggcattgcatttaaaatatatgagggttctaaaaatttttatccttgcgttgaaataaaggcttctcccgcaaaagtattacagggtcataatgtttttggtacaaccgatttagctttatgctctgaggctttattgcttaattttgctaattctttgccttgcctgtatgatttattggatgttggaatcgcctgatgcggtattttctccttacgcatctgtgcggtatttcacaccgcatatggtgcactctcagtacaatctgctctgatgccgcatagttaagccagccccgacacccgccaacacccgctgacgcgccctgacgggcttgtctgctcccggcatccgcttacagacaagctgtgaccgtctccgggagctgcatgtgtcagaggttttcaccgtcatcaccgaaacgcgcgagacgaaagggcctcgtgatacgcctatttttataggttaatgtcatgataataatggtttcttagacgtcaggtggcacttttcggggaaatgtgcgcggaacccctatttgtttatttttctaaatacattcaaatatgtatccgctcatgagacaataaccctgataaatgcttcaataatattgaaaaaggaagagtatgattgaacaagatggattgcacgcaggttctccggccgcttgggtggagaggctattcggctatgactgggcacaacagacaatcggctgctctgatgccgccgtgttccggctgtcagcgcaggggcgcccggttctttttgtcaagaccgacctgtccggtgccctgaatgaactgcaagacgaggcagcgcggctatcgtggctggccacgacgggcgttccttgcgcagctgtgctcgacgttgtcactgaagcgggaagggactggctgctattgggcgaagtgccggggcaggatctcctgtcatctcaccttgctcctgccgagaaagtatccatcatggctgatgcaatgcggcggctgcatacgcttgatccggctacctgcccattcgaccaccaagcgaaacatcgcatcgagcgagcacgtactcggatggaagccggtcttgtcgatcaggatgatctggacgaagagcatcaggggctcgcgccagccgaactgttcgccaggctcaaggcgagcatgcccgacggcgaggatctcgtcgtgacccatggcgatgcctgcttgccgaatatcatggtggaaaatggccgcttttctggattcatcgactgtggccggctgggtgtggcggaccgctatcaggacatagcgttggctacccgtgatattgctgaagagcttggcggcgaatgggctgaccgcttcctcgtgctttacggtatcgccgctcccgattcgcagcgcatcgccttctatcgccttcttgacgagttcttctgactgtcagaccaagtttactcatatatactttagattgatttaaaacttcatttttaatttaaaaggatctaggtgaagatcctttttgataatctcatgaccaaaatcccttaacgtgagttttcgttccactgagcgtcagaccccgtagaaaagatcaaaggatcttcttgagatcctttttttctgcgcgtaatctgctgcttgcaaacaaaaaaaccaccgctaccagcggtggtttgtttgccggatcaagagctaccaactctttttccgaaggtaactggcttcagcagagcgcagataccaaatactgttcttctagtgtagccgtagttaggccaccacttcaagaactctgtagcaccgcctacatacctcgctctgctaatcctgttaccagtggctgctgccagtggcgataagtcgtgtcttaccgggttggactcaagacgatagttaccggataaggcgcagcggtcgggctgaacggggggttcgtgcacacagcccagcttggagcgaacgacctacaccgaactgagatacctacagcgtgagctatgagaaagcgccacgcttcccgaagggagaaaggcggacaggtatccggtaagcggcagggtcggaacaggagagcgcacgagggagcttccagggggaaacgcctggtatctttatagtcctgtcgggtttcgccacctctgacttgagcgtcgatttttgtgatgctcgtcaggggggcggagcctatggaaaaacgccagcaacgcggcctttttacggttcctggccttttgctggccttttgctcacatgttctttcctgcgttatcccctgattctgtggataaccgtattaccgcctttgagtgagctgataccgctcgccgcagccgaacgaccgagcgcagcgagtcagtgagcgaggaagcggaagagcgcccaatacgcaaaccgcctctccccgcgcgttggccgattcattaatgcagctgcgcgctcgctcgctcactgaggccgcccgggcaaagcccgggcgtcgggcgacctttggtcgcccggcctcagtgagcgagcgagcgcgcagagagggagtggccaactccatcactaggggttccttgtagttaatgattaacccgccatgctacttatctacgtagccatgctctagcggcctcggcctctgcataaataaaaaaaattagtcagccatgagcttggcccattgcatacgttgtatccatatcataatatgtacatttatattggctcatgtccaacattac

SEQ ID NO: 6 - DNA, 20 bp, synthetic construct
  source 1..20: mol_type = other DNA
gtggcactgaccaagacgta

SEQ ID NO: 7 - DNA, 20 bp, synthetic construct
  source 1..20: mol_type = other DNA
ctgacgtcctcatgtaggcc

SEQ ID NO: 8 - DNA, 20 bp, synthetic construct
  source 1..20: mol_type = other DNA
tcctccattctccctcctcg

SEQ ID NO: 9 - DNA, 20 bp, synthetic construct
  source 1..20: mol_type = other DNA
cgaattggctctgacctggt

SEQ ID NO: 10 - DNA, 20 bp, synthetic construct
  source 1..20: mol_type = other DNA
gagcttgaactggtgctcca

SEQ ID NO: 11 - DNA, 20 bp, synthetic construct
  source 1..20: mol_type = other DNA
tctcaacagtaggtgcctgc

SEQ ID NO: 12 - DNA, 669 bp, synthetic construct
  source 1..669: mol_type = other DNA
atggcagcaaggcccaagctccactatcccaacggaagaggccggatggagtccgtgagatgggttttagctgccgccggagtcgagtttgatgaagaatttctggaaacaaaagaacagttgtacaagttgcaggatggtaaccacctgctgttccaacaagtgcccatggttgaaattgacgggatgaagttggtacagacccgaagcattctccactacatagcagacaagcacaatctctttggcaagaacctcaaggagagaaccctgattgacatgtacgtggaggggacactggatctgctggaactgcttatcatgcatcctttcttaaaaccagatgatcagcaaaaggaagtggttaacatggcccagaaggctataattagatactttcctgtgtttgaaaagattttaaggggtcacggacaaagctttcttgttggtaatcagctgagccttgcagatgtgattttactccaaaccattttagctctagaagagaaaattcctaatatcctgtctgcatttcctttcctccaggaatacacagtgaaactaagtaatatccctacaattaagagattccttgaacctggcagcaagaagaagcctccccctgatgaaatttatgtgagaaccgtctacaacatctttaggccataa

SEQ ID NO: 13 - protein, 401 aa, synthetic construct
MEKSKNFRIDALLAVDPPRAASAQSAPLALVTSLAAAASGTGGGGGGGGASGGTSGSCSPASSEPPAAPADRLRAESPSPPRLLAAHCALLPKPGFLGAGGGGGGTGGGHGGPHHHAHPGAAAAAAAAAAAAAAGGLALGLHPGGAQGGAGLPAQAALYGHPVYGYSAAAAAAALAGQHPALSYSYPQVQGAHPAHPADPIKLGAGTFQLDQWLRASTAGMILPKMPDFNSQAQSNLLGKCRRPRTAFTSQQLLELEHQFKLNKYLSRPKRFEVATSLMLTETQVKIWFQNRRMKWKRSKKAKEQAAQEAEKQKGGGGGAGKGGAEEPGAEELLGPPAPGDKGSGRRLRDLRDSDPEEDEDEDDEDHFPYSNGASVHAASSDCSSEDDSPPPRPSHQPAPQ

SEQ ID NO: 14 - DNA, 1203 bp, synthetic construct
  source 1..1203: mol_type = other DNA
atggaaaaatccaaaaatttccgcatcgacgccctgctggcggtggaccccccacgagccgcctctgcgcagagcgcgccgctggccttggtcacgtcgctcgccgccgccgcatctggcaccggaggtggcggcggcggcggcggggcgagcggcgggactagcggcagctgcagccccgcgtcctcggagccgccggctgcgcccgccgaccgcctgcgcgccgagagcccgtcgccgccgcgcctgctggccgcgcactgcgcgctgctgcccaagccgggcttcctgggcgcgggcggcggcggcggcggcacgggcggcgggcacggggggccccaccaccacgcgcatccgggcgcagcggccgctgccgccgccgccgccgccgccgccgccgctgggggcctggcgctggggctgcaccctgggggcgcgcagggcggcgcgggcctcccggcgcaggcggcgctctacggccacccggtctacggctactccgcggcggcggcggcggctgcgctggcgggccagcacccggcgctctcctactcgtacccgcaggtgcaaggcgcgcaccccgcgcaccccgccgaccccatcaagctgggcgccggcaccttccagctggaccagtggctgcgcgcgtccaccgcgggcatgatcctgcctaagatgcccgacttcaactcccaggcgcagtcgaacctcctggggaagtgccgccggccgcgcaccgccttcaccagccagcagctgctggagctggagcaccagttcaagctcaacaagtacctgtcgcggcccaagcgcttcgaggtggccacctcgctcatgctcaccgagacccaggtgaagatttggttccagaaccggcggatgaaatggaaacgcagcaaaaaggccaaagagcaggcggcgcaggaagcggagaaacagaagggcggcggcgggggcgcggggaagggcggcgcggaggagccgggagccgaggagctgctggggccgccagcgcccggagacaagggcagcggacgccgcctgcgggacttgagggacagtgaccccgaggaggacgaggacgaggacgacgaggaccatttcccctacagcaacggcgccagcgtccacgccgcctcctccgactgctcctcggaggacgactcgccgcccccgcggcccagccaccagcccgcgccccag

SEQ ID NO: 15 - protein, 402 aa, synthetic construct
MEARGELGPARESAGGDLLLALLARRADLRREIPLCAGCDQHILDRFILKALDRHWHSKCLKCSDCHTPLAERCFSRGESVYCKDDFFKRFGTKCAACQLGIPPTQVVRRAQDFVYHLHCFACVVCKRQLATGDEFYLMEDSRLVCKADYETAKQREAEATAKRPRTTITAKQLETLKSAYNTSPKPARHVREQLSSETGLDMRVVQVWFQNRRAKEKRLKKDAGRQRWGQYFRNMKRSRGGSKSDKDSVQEGQDSDAEVSFPDEPSLAEMGPANGLYGSLGEPTQALGRPSGALGNFSLEHGGLAGPEQYRELRPGSPYGVPPSPAAPQSLPGPQPLLSSLVYPDTSLGLVPSGAPGGPPPMRVLAGNGPSSDLSTGSSGGYPDFPASPASWLDEVDHAQF

SEQ ID NO: 16 - DNA, 1206 bp, synthetic construct
  source 1..1206: mol_type = other DNA
atggaagccagaggcgaactgggccctgccagagaatctgccggcggagatctgctgctggccctgctggctagaagggccgacctgagaagagaaatccccctgtgcgccggctgcgaccagcacatcctggaccggtttatcctgaaggccctggacagacactggcacagcaagtgcctgaagtgcagcgactgccacacccccctggccgagagatgctttagcagaggcgagagcgtgtactgcaaggacgacttcttcaagagattcggcaccaagtgcgccgcctgccagctgggaattcctcctacacaggtcgtgcggagagcccaggacttcgtgtaccatctgcactgcttcgcctgcgtcgtgtgcaagagacagctggccaccggcgacgagttctacctgatggaagatagccggctcgtgtgtaaagccgactacgagacagccaagcagagagaggccgaggccaccgccaaaagacccagaaccaccatcaccgccaagcagctggaaaccctgaagtccgcctacaacaccagccccaagcccgccagacatgtgcgggaacagctgagcagcgagacaggcctggacatgagagtggtgcaagtgtggttccagaacagacgggccaaagagaagcggctgaagaaggacgccggcaggcagagatggggccagtacttccggaacatgaagcggtccagaggcggcagcaagagcgacaaggacagcgtgcaggaaggccaggacagcgacgccgaggtgtccttcccagatgagcctagcctggccgaaatgggcccagccaatggcctgtatggcagcctgggagagccaacccaggctctgggcagaccttctggcgccctgggcaacttctctctggaacacggcggactggccggacccgagcagtatagagaactgaggcccggcagcccttacggcgtgccaccttctccagctgcccctcagtctctgccaggacctcagcctctgctgtccagcctggtgtaccccgatacaagcctgggcctggtgccatctggcgctccaggcggacctcctccaatgagagtgctggccggcaatggccctagcagcgatctgagcacaggcagctctggcggctaccccgattttcctgccagccctgcctcctggctggacgaagtggatcacgcccagttc

SEQ ID NO: 17 - protein, 231 aa, synthetic construct
MESSGKMESGAGQQPQPPQPFLPPAACFFATAAAAAAAAAAAAQSAQQQQPQAPPQQAPQLSPVADSQPSGGGHKSAAKQVKRQRSSSPELMRCKRRLNFSGFGYSLPQQQPAAVARRNERERNRVKLVNLGFATLREHVPNGAANKKMSKVETLRSAVEYIRALQQLLDEHDAVSAAFQAGVLSPTISPNYSNDLNSMAGSPVSSYSSDEGSYDPLSPEEQELLDFTNWF

SEQ ID NO: 18 - DNA, 696 bp, synthetic construct
  source 1..696: mol_type = other DNA
atggagagctctggcaagatggagagtggagccggccagcagccgcagcccccgcagcccttcctgcctcccgcagcctgcttctttgcgaccgcggcggcggcggcagcggcggcggccgcggcagctcagagcgcgcagcagcaacagccgcaggcgccgccgcagcaggcgccgcagctgagcccggtggccgacagccagccctcagggggcggtcacaagtcagcggccaagcaggtcaagcgccagcgctcgtcctctccggaactgatgcgctgcaaacgccggctcaacttcagcggcttcggctacagcctgccacagcagcagccggccgccgtggcgcgccgcaacgagcgcgagcgcaaccgggtcaagttggtcaacctgggttttgccaccctccgggagcatgtccccaacggcgcggccaacaagaagatgagcaaggtggagacgctgcgctcggcggtcgagtacatccgcgcgctgcagcagctgctggacgagcacgacgcggtgagcgctgcctttcaggcgggcgtcctgtcgcccaccatctcccccaactactccaacgacttgaactctatggcgggttctccggtctcgtcctactcctccgacgagggatcctacgaccctcttagcccagaggaacaagagctgctggactttaccaactggttctga

SEQ ID NO: 19 - protein, 284 aa, synthetic construct
MATAASNHYSTSSASVHAGGMGAGGYRASVGDYGASNGHSHAHWTASHGGGGGGGGGGGGGGGGGGGGGDGSWSTSGDKSVVVGGRGDHGGAHRHVHHAANHHGGAWRSAAAAAHSMGASNGGYSSTVNGMGAGGAGHHHGRDAHDHHADHHHHSHHGGHGAHHDHSDDTTSDDAKKRRKGTADVGAGTYGNVSTTCRASKNMCKKNKWADSSSGSTSDKAAGRKRKKRTSVSVKGASHKCKSATSADSKVVRVWCNRRKKRMTGGTGADVYGGSRDTHHGVTV

SEQ ID NO: 20 - DNA, 1338 bp, synthetic construct
  source 1..1338: mol_type = other DNA
atggcgaccgcagcgtctaaccactacagcctgctcacctccagcgcctccatcgtacatgccgagccgcctggcggcatgcagcagggcgcagggggctaccgcgaggcgcagagcctggtgcagggcgactacggcgcgctgcagagcaacgggcacccgctcagccacgctcaccagtggatcaccgcgctgtcccacggcggcggcggcgggggcggcggcggcggtggaggaggcgggggaggcggcgggggaggcggcgacggctccccgtggtccaccagccccctaggccagccggacatcaagccctcggtggtggtacagcagggtggccgaggcgacgagctgcacgggccaggagcgctgcagcaacagcatcaacagcaacagcaacagcagcagcagcagcagcagcagcagcagcagcaacagcagcagcaacaacagcgaccgccacatctggtgcaccacgctgccaaccaccatcccgggcccggggcatggcggagtgcggcggctgcagctcacctccctccctccatgggagcttccaacggcggtttgctctattcgcagccgagcttcacggtgaacggcatgctgggcgcaggagggcagccggctgggctgcaccaccacggcctgagggacgcccacgatgagccacaccatgcagaccaccacccgcatccgcactctcacccacaccagcaaccgcccccgccacctcccccacaaggcccaccgggccacccaggcgcgcaccacgacccgcactcggacgaggacacgccgacctcagacgacctggagcagttcgccaagcaattcaagcagaggcggatcaaactcggatttactcaagcagacgtggggctggcgcttggcaccctgtacggcaacgtgttctcgcagaccaccatctgcaggtttgaggccctgcagctgagcttcaagaacatgtgcaagctgaagcctttgttgaacaagtggttggaagaggcagactcatcctcgggcagccccaccagcatagacaagatcgcagcgcaagggcgcaaacggaaaaagcggacctccatcgaggtgagcgtcaagggggctctggagagccatttcctcaaatgccctaagccctcggcccaggagatcacctccctcgcggacagcttacagctggagaaggaggtggtgagagtttggttttgtaacaggagacagaaagagaaaaggatgacccctcccggagggactctgccgggcgccgaggatgtgtatgggggtagtagggacacgccaccacaccacggggtgcagacgcccgtccagtga

SEQ ID NO: 21 - protein, 813 aa, synthetic construct
MDVDSKRHRTRSKGVRVVASCTGCDGSGHVSGKYARHRSVYGCAKKRKTDKAKRKAVKADSSSVDCYSDGTDMDDKDDDSDNDGDDDDDVDRDDDDDDDDGDDVDDDNDHMSCTRMDTDKDDNNNDYDNYDVAKSNGKADAAYRARTSMNSNTSNSDDSDKNNGRKSSDDSDVVRTVDSKAGHGVVSNSDRSYAGMSDSRNMNYVMGKMNNGMKMVSDVCSSCRNCDARKSTNDRSNMSVRHVRDDGRTDRSYSDMMNMRSRSRTSSCAKDGCHRDDDTTSVNSDRSVDMTKGNTKAATRAKAMRKMAMDAGRRDNRSYDSRAGDRKSKSSDSHVKKYYGKDSRTKRSKCTGCDGTGHVTGYHHRSSGCHKDRVAMHNVKCTGCTGRGHVNSNRNSHRSSGCAAAKAKAKHSCDVSKSNASDRVRMCVKYGYRNNVTTTRSNAKKYSKTSYNSYDNHTYGKRAAKVTRDSKGYDDAKRYCKNASSSSTTSSYASSSSNSCGGGSSASSTCSKSSDYTHDMAAHMAATANSTRCRMNSTKDCTARNDMVDNGTDSMNKRRDSCCVTMSAVMSSRCSGDCWDVDYTKMKRRVDDKTDDARRYGVTSKKYCKSKKDTSGCADKSRSMATSSKCTGCDGSGHTGNYASHRSSGCRAKKSGRASKDKDRCVGCDGGHTGKYASHRSASGCAAKRKDGYNGSSWKSVKTGMSCTGCDGSGHVSGSTHRSSGCRATSAMKKAKSGMTKRASNGNDKDKNSNSMADMKRTTTMSNKTNKVNSHANSSHSANHMDNNDAYVTTTMYTNDRYSNKANKAVRGV

SEQ ID NO: 22 - DNA, 3564 bp, synthetic construct
  source 1..3564: mol_type = other DNA
atggacgtggactctgaggagaagcgccatcgcacacggtccaaaggggttcgagttcctgtggagccagccatacaagagctgttcagctgtcccactccaggctgcgacggcagtggtcacgtcagtggcaaatatgcacgacacagaagtgtatatggttgtcccttggctaaaaaaagaaaaacgcaagataaacagccccaagaacctgctcccaagcgaaaaccatttgcagtaaaagcagatagttcctcagtagacgaatgttatgagagtgatggtactgaagacatggatgataaggaggaagatgatgatgaggagttctctgaagacaatgatgagcaaggggatgatgacgacgaagatgaggtggatcgggaagacgaggaggagatcgaggaggaagatgatgaagaagatgatgatgatgaagatggtgacgatgtagaagaggaagaagaggatgatgatgaagaggaggaagaagaggaagaggaagaagaaaatgaagaccatcaaatgagttgtactcgaataatgcaggacacagacaaggatgataacaacaatgatgagtatgataactatgatgaactggtagctaagtcgctattaaatcttggcaaaattgctgaggatgcagcataccgagccaggactgaatcagagatgaacagcaatacctccaatagtctggaggacgatagtgacaaaaacgaaaacctcggtcggaaaagcgaactgagtctagacttagacagtgatgttgttagagaaacagtggactcccttaagctgttagcacaaggacatggtgttgtgctatcagagaatatcagtgacagaagttatgctgaggggatgtcacagcaggacagtagaaatatgaactatgtcatgctagggaagcccatgaacaatggactcatggagaagatggtggaggagagtgatgaggaagtgtgtctaagtagtctagagtgcctgaggaaccagtgctttgacctggccaggaaactcagcgagaccaacccacaggacaggagtcagccacccaacatgagtgtgcgccaacatgtccggcaagaggacgacttccctgggaggacgccagacaggagctactcggatatgatgaaccttatgcggctggaggagcagctcagtcccaggtctagaacgttctccagctgtgccaaggaggatgggtgtcatgagagggatgatgacaccacctcagtgaactcagacaggtctgaggaagtgtttgacatgaccaagggcaacctgactctgctagagaaagccattgccttggagacagagagagccaaggccatgcgggagaagatggccatggatgctgggagaagggataacctgagatcctatgaggaccagtctccaagacagctggctggggaagacagaaaatccaaatccagtgacagccatgtcaaaaagccatactatggtaaagatccctcaagaacagaaaagagagagagcaagtgtccaacccccgggtgtgatggaaccggccacgtaactgggctttacccgcatcaccgcagtctgtctggatgcccgcacaaagatagggtccctccagaaattcttgccatgcatgaaaatgttctcaagtgtcccactccaggctgcacagggcgagggcatgtgaatagcaacaggaactcgcacagaagcctctctggatgccccattgctgctgcagaaaaactggcaaaggcccaagagaaacaccagagctgtgatgtgtccaaatccaaccaggcctcagaccgagtcctcaggccaatgtgctttgtcaaacagcttgagattcctcagtatggctacagaaacaatgttcccacaaccacaccacgctccaacctggccaaggagcttgagaaatactccaagacttcgtttgagtacaacagttacgacaaccatacttatggcaaaagagccatagctcccaaggtgcaaaccagggacatatcccccaaaggatatgacgatgccaagcggtactgcaagaatgccagccccagcagcagcaccaccagcagctatgcacctagcagcagcagcaacctcagctgtggtggtggcagcagcgccagtagcacgtgtagcaagagcagctttgactacacacatgacatggaggccgcacacatggcagccacagccattctcaacctgtccacacgttgtcgtgaaatgccacagaacctgtccaccaagccacaggacctgtgtactgcccggaacccagacatggaggtggatgagaatggcaccctggacctgagcatgaacaagcagaggcctcgagacagctgctgcccagtcctgacacccctggaacccatgtctccgcagcagcaggccgtgatgagcagccgatgcttccagctgagcgagggggattgctgggacttgcctgtagactacaccaaaatgaagcctcggagggtagatgaggatgagcccaaagagattaccccagaagacttggacccattccaggaggctctggaagaaagacggtatccaggggaggtgaccatcccaagccccaaacccaagtaccctcagtgcaaggaaagcaaaaaggacttaataactctgtctggctgccccctggcggacaaaagcattcgaagtatgctggccaccagttcccaagagctcaagtgccccacccctggctgtgacggttctggacacatcactggcaattacgcttctcatcgaagcctttctgggtgcccgagagcaaagaagagtggcatccggatagcacagagcaaagaggacaaggaagaccaggagccaatcaggtgtccggtacctggctgtgacggtcagggacacatcactgggaagtatgcatcccaccgcagcgcctccgggtgtcccttggcagccaagaggcagaaagatgggtaccttaatggctcccagttctcctggaagtcggtcaagacggagggcatgtcctgccctacccccgggtgtgatgggtcaggacacgtcagtggcagcttcctcacacaccgcagcttgtcaggatgtccaagagccacatcagcaatgaagaaagcaaagctgtctggagaacagatgttgactatcaagcagcgagccagcaacggtatagaaaatgatgaagaaatcaagcagttagatgaagagatcaaggagcttaatgagtccaattcccagatggaggctgacatgatcaaactcagaactcagatcaccacaatggagagcaacctgaagacgattgaggaggagaacaaagtcattgaacagcagaatgagtcgctcttgcacgagttggccaacctgagccagtccctgatccacagcctcgccaacatccagctgcctcacatggatccaatcaatgaacaaaattttgatgcttacgtgactactttgacggaaatgtatacaaatcaagatcgttatcagagtccagaaaataaagccctactggaaaatataaagcaggctgtgagaggaattcaggtctga

SEQ ID NO: 23 - protein, 231 aa, synthetic construct
MGDMGDKKKRSCVGCGNHDYRVSDWHAACKCACNYDSCTCVRDGKTYCKRDYRYGKCAKCSGSKNDVMRARSKVYHCRCVACSRGDARDGCRADHDVVRASGAGDSHARMAASARARHVHKKTTRVRTVNKHTRTCYAANRDAMKVMTGSRVRVWNKRCKDKKRSMMKNDKTNGMTGTMVAASRHDGGANVVSYWKVSDASDDAVNSGGGSNSTGSVASMSSDTNSMVASA

SEQ ID NO: 24 - DNA, 1050 bp, synthetic construct
  source 1..1050: mol_type = other DNA
atgggagacatgggcgatccaccaaaaaaaaaacgtctgatttccctgtgtgttggttgcggcaatcaaattcacgaccagtatattctgagggtttctccggatttggagtggcatgcagcatgtttgaaatgtgcggagtgtaatcagtatttggacgaaagctgtacgtgctttgttagggatgggaaaacctactgtaaaagagattatatcaggttgtacgggatcaaatgcgccaagtgcagcataggcttcagcaagaacgacttcgtgatgcgtgcccgctctaaggtgtaccacatcgagtgtttccgctgtgtagcctgcagccgacagctcatcccgggagacgaattcgccctgcgggaggatgggcttttctgccgtgcagaccacgatgtggtggagagagccagcctgggagctggagaccctctcagtcccttgcatccagcgcggcctctgcaaatggcagccgaacccatctcggctaggcagccagctctgcggccgcacgtccacaagcagccggagaagaccacccgagtgcggactgtgctcaacgagaagcagctgcacaccttgcggacctgctatgccgccaaccctcggccagatgcgctcatgaaggagcaactagtggagatgacgggcctcagtcccagagtcatccgagtgtggtttcaaaacaagcggtgcaaggacaagaaacgcagcatcatgatgaagcagctccagcagcagcaacccaacgacaaaactaatatccaggggatgacaggaactcccatggtggctgctagtccggagagacatgatggtggtttacaggctaacccagtagaggtgcaaagttaccagccgccctggaaagtactgagtgacttcgccttgcaaagcgacatagatcagcctgcttttcagcaactggtcaatttttcagaaggaggaccaggctctaattctactggcagtgaagtagcatcgatgtcctcgcagctcccagatacacccaacagcatggtagccagtcctattgaggcatga

SEQ ID NO: 25 - protein, 178 aa, synthetic construct
MVKSTKVMGSASASATTMSSSADDRRGSARGRGAAGGVGSASGAGGCRGRGMHCKRRSRSRAVSRGAKTATVRKKTRRKANNRRNRMHNNAADARVTDAKTKTRAHNYWATTRADHCAGAGGGATAVSGAAGASGDSSSSWSCTNSASSSNSTSYSCTSASGSDVDYWKHRYAHARDC

SEQ ID NO: 26 - DNA, 792 bp, synthetic construct
  source 1..792: mol_type = other DNA
atgttcgtcaaatctgagactctggagttgaaggaggaagaggaggtactgatgctgctgggctcggcttccccggcctcggcgaccctgaccccgatgtcctccagcgcggacgaggaggaggacgaggagctgcgccggccgggctccgcgcgtgggcagcgtggagcggaagccgggcagggggtgcagggcagtccggcgtcgggtgccgggggttgccggccagggcggctgctgggcctgatgcacgagtgcaagcgtcgcccgtcgcgctcacgggccgtctcccgaggtgccaagacggcggagacggtgcagcgcatcaagaagacccgcaggctcaaggccaacaaccgcgagcgcaaccgcatgcacaacctaaacgccgcgctggacgcgctgcgcgaggtgctgcccaccttccccgaggatgccaagctcacgaagatcgagacgctgcgcttcgcccacaattacatctgggcgctcaccgagactctgcgcctggcggaccactgcgccggcgccggtggcctccagggggcgctcttcacggaggcggtgctcctgagcccgggagctgcgctcggcgccagcggggacagcccttctccaccttcctcctggagctgcaccaacagcccggcgtcatcctccaactccacgtccccatacagctgcactttatcgcccgctagccccgggtcagacgtggactactggcagcccccacctccggagaagcatcgttatgcgcctcacctgcccctcgccagggactgtatctag

SEQ ID NO: 27 - protein, 216 aa, synthetic construct
MTKSYSSGMGGSWTDCSSDHADKKDAMNADSRNGGDDDKKRRGKKKKMTKARRKRRMKANARRNRMHGNAADNRKVVCYSKTKSKTRAKNYWASRSGKSDVSVTCKGSTTNVAGCNRTNDMHTASASVHYSYSGSYGTMDSSHVHVKHAYSAASTDCTSSDGSSNGNSKHSAKNYATMHYAATAGSHGSSSGAAARCDNMSDSHSHHRVMSANAHD

SEQ ID NO: 28 - DNA, 1074 bp, synthetic construct
  source 1..1074: mol_type = other DNA
atgaccaaatcatacagcgagagcgggctgatgggcgagcctcagccccaaggtcccccaagctggacagatgagtgtctcagttctcaggacgaggaacacgaggcagacaagaaagaggacgagcttgaagccatgaatgcagaggaggactctctgagaaacgggggagaggaggaggaggaagatgaggatctagaggaagaggaggaagaagaagaggaggaggaggatcaaaagcccaagagacggggtcccaaaaagaaaaagatgaccaaggcgcgcctagaacgttttaaattaaggcgcatgaaggccaacgcccgcgagcggaaccgcatgcacgggctgaacgcggcgctggacaacctgcgcaaggtggtaccttgctactccaagacccagaaactgtctaaaatagagacactgcgcttggccaagaactacatctgggctctgtcagagatcctgcgctcaggcaaaagccctgatctggtctccttcgtacagacgctctgcaaaggtttgtcccagcccactaccaatttggtcgccggctgcctgcagctcaaccctcggactttcttgcctgagcagaacccggacatgcccccgcatctgccaaccgccagcgcttccttcccggtgcatccctactcctaccagtcccctggactgcccagcccgccctacggcaccatggacagctcccacgtcttccacgtcaagccgccgccacacgcctacagcgcagctctggagcccttctttgaaagccccctaactgactgcaccagcccttcctttgacggacccctcagcccgccgctcagcatcaatggcaacttctctttcaaacacgaaccatccgccgagtttgaaaaaaattatgcctttaccatgcactaccctgcagcgacgctggcagggccccaaagccacggatcaatcttctcttccggtgccgctgcccctcgctgcgagatccccatagacaacattatgtctttcgatagccattcgcatcatgagcgagtcatgagtgcccagcttaatgccatctttcacgattag

SEQ ID NO: 29 - DNA, 6952 bp, synthetic construct
  source 1..6952: mol_type = other DNA
cctgcaggcagctgcgcgctcgctcgctcactgaggccgcccgggcaaagcccgggcgtcgggcgacctttggtcgcccggcctcagtgagcgagcgagcgcgcagagagggagtggccaactccatcactaggggttccttctagacaactttgtatagaaaagttgtagttattaatagtaatcaattacggggtcattagttcatagcccatatatggagttccgcgttacataacttacggtaaatggcccgcctggctgaccgcccaacgacccccgcccattgacgtcaataatgacgtatgttcccatagtaacgccaatagggactttccattgacgtcaatgggtggagtatttacggtaaactgcccacttggcagtacatcaagtgtatcatatgccaagtacgccccctattgacgtcaatgacggtaaatggcccgcctggcattatgcccagtacatgaccttatgggactttcctacttggcagtacatctacgtattagtcatcgctattaccatggtgatgcggttttggcagtacatcaatgggcgtggatagcggtttgactcacggggatttccaagtctccaccccattgacgtcaatgggagtttgttttggcaccaaaatcaacgggactttccaaaatgtcgtaacaactccgccccattgacgcaaatgggcggtaggcgtgtacggtgggaggtctatataagcagagctggtttagtgaaccgtcagatccaagtttgtacaaaaaagcaggctgccaccatggaaaaatccaaaaatttccgcatcgacgccctgctggcggtggaccccccacgagccgcctctgcgcagagcgcgccgctggccttggtcacgtcgctcgccgccgccgcatctggcaccggaggtggcggcggcggcggcggggcgagcggcgggactagcggcagctgcagccccgcgtcctcggagccgccggctgcgcccgccgaccgcctgcgcgccgagagcccgtcgccgccgcgcctgctggccgcgcactgcgcgctgctgcccaagccgggcttcctgggcgcgggcggcggcggcggcggcacgggcggcgggcacggggggccccaccaccacgcgcatccgggcgcagcggccgctgccgccgccgccgccgccgccgccgccgctgggggcctggcgctggggctgcaccctgggggcgcgcagggcggcgcgggcctcccggcgcaggcggcgctctacggccacccggtctacggctactccgcggcggcggcggcggctgcgctggcgggccagcacccggcgctctcctactcgtacccgcaggtgcaaggcgcgcaccccgcgcaccccgccgaccccatcaagctgggcgccggcaccttccagctggaccagtggctgcgcgcgtccaccgcgggcatgatcctgcctaagatgcccgacttcaactcccaggcgcagtcgaacctcctggggaagtgccgccggccgcgcaccgccttcaccagccagcagctgctggagctggagcaccagttcaagctcaacaagtacctgtcgcggcccaagcgcttcgaggtggccacctcgctcatgctcaccgagacccaggtgaagatttggttccagaaccggcggatgaaatggaaacgcagcaaaaaggccaaagagcaggcggcgcaggaagcggagaaacagaagggcggcggcgggggcgcggggaagggcggcgcggaggagccgggagccgaggagctgctggggccgccagcgcccggagacaagggcagcggacgccgcctgcgggacttgagggacagtgaccccgaggaggacgaggacgaggacgacgaggaccatttcccctacagcaacggcgccagcgtccacgccgcctcctccgactgctcctcggaggacgactcgccgcccccgcggcccagccaccagcccgcgccccagggtagcggtgccactaacttctccctgttgaaacaagcaggggatgtcgaagagaatcctggtccaatggaagccagaggcgaactgggccctgccagagaatctgccggcggagatctgctgctggccctgctggctagaagggccgacctgagaagagaaatccccctgtgcgccggctgcgaccagcacatcctggaccggtttatcctgaaggccctggacagacactggcacagcaagtgcctgaagtgcagcgactgccacacccccctggccgagagatgctttagcagaggcgagagcgtgtactgcaaggacgacttcttcaagagattcggcaccaagtgcgccgcctgccagctgggaattcctcctacacaggtcgtgcggagagcccaggacttcgtgtaccatctgcactgcttcgcctgcgtcgtgtgcaagagacagctggccaccggcgacgagttctacctgatggaagatagccggctcgtgtgtaaagccgactacgagacagccaagcagagagaggccgaggccaccgccaaaagacccagaaccaccatcaccgccaagcagctggaaaccctgaagtccgcctacaacaccagccccaagcccgccagacatgtgcgggaacagctgagcagcgagacaggcctggacatgagagtggtgcaagtgtggttccagaacagacgggccaaagagaagcggctgaagaaggacgccggcaggcagagatggggccagtacttccggaacatgaagcggtccagaggcggcagcaagagcgacaaggacagcgtgcaggaaggccaggacagcgacgccgaggtgtccttcccagatgagcctagcctggccgaaatgggcccagccaatggcctgtatggcagcctgggagagccaacccaggctctgggcagaccttctggcgccctgggcaacttctctctggaacacggcggactggccggacccgagcagtatagagaactgaggcccggcagcccttacggcgtgccaccttctccagctgcccctcagtctctgccaggacctcagcctctgctgtccagcctggtgtaccccgatacaagcctgggcctggtgccatctggcgctccaggcggacctcctccaatgagagtgctggccggcaatggccctagcagcgatctgagcacaggcagctctggcggctaccccgattttcctgccagccctgcctcctggctggacgaagtggatcacgcccagttcggcagtggagagggcagaggaagtctgctaacatgcggtgacgtcgaggagaatcctggcccaatggcagcaaggcccaagctccactatcccaacggaagaggccggatggagtccgtgagatgggttttagctgccgccggagtcgagtttgatgaagaatttctggaaacaaaagaacagttgtacaagttgcaggatggtaaccacctgctgttccaacaagtgcccatggttgaaattgacgggatgaagttggtacagacccgaagcattctccactacatagcagacaagcacaatctctttggcaagaacctcaaggagagaaccctgattgacatgtacgtggaggggacactggatctgctggaactgcttatcatgcatcctttcttaaaaccagatgatcagcaaaaggaagtggttaacatggcccagaaggctataattagatactttcctgtgtttgaaaagattttaaggggtcacggacaaagctttcttgttggtaatcagctgagccttgcagatgtgattttactccaaaccattttagctctagaagagaaaattcctaatatcctgtctgcatttcctttcctccaggaatacacagtgaaactaagtaatatccctacaattaagagattccttgaacctggcagcaagaagaagcctccccctgatgaaatttatgtgagaaccgtctacaacatctttaggccataaacccagctttcttgtacaaagtgggaattcctagagctcgctgatcagcctcgactgtgccttctagttgccagccatctgttgtttgcccctcccccgtgccttccttgaccctggaaggtgccactcccactgtcctttcctaataaaatgaggaaattgcatcgcattgtctgagtaggtgtcattctattctggggggtggggtggggcaggacagcaagggggaggattgggaagagaatagcaggcatgctggggagggccgcaggaacccctagtgatggagttggccactccctctctgcgcgctcgctcgctcactgaggccgggcgaccaaaggtcgcccgacgcccgggctttgcccgggcggcctcagtgagcgagcgagcgcgcagctgcctgcaggggcgcctgatgcggtattttctccttacgcatctgtgcggtatttcacaccgcatacgtcaaagcaaccatagtacgcgccctgtagcggcgcattaagcgcggcgggtgtggtggttacgcgcagcgtgaccgctacacttgccagcgccttagcgcccgctcctttcgctttcttcccttcctttctcgccacgttcgccggctttccccgtcaagctctaaatcgggggctccctttagggttccgatttagtgctttacggcacctcgaccccaaaaaacttgatttgggtgatggttcacgtagtgggccatcgccctgatagacggtttttcgccctttgacgttggagtccacgttctttaatagtggactcttgttccaaactggaacaacactcaactctatctcgggctattcttttgatttataagggattttgccgatttcggtctattggttaaaaaatgagctgatttaacaaaaatttaacgcgaattttaacaaaatattaacgtttacaattttatggtgcactctcagtacaatctgctctgatgccgcatagttaagccagccccgacacccgccaacacccgctgacgcgccctgacgggcttgtctgctcccggcatccgcttacagacaagctgtgaccgtctccgggagctgcatgtgtcagaggttttcaccgtcatcaccgaaacgcgcgagacgaaagggcctcgtgatacgcctatttttataggttaatgtcatgataataatggtttcttagacgtcctggcccgtgtctcaaaatctctgatgttacattgcacaagataaaaatatatcatcatgaacaataaaactgtctgcttacataaacagtaatacaaggggtgttatgagccatattcaacgggaaacgtcgaggccgcgattaaattccaacatggatgctgatttatatgggtataaatgggctcgcgataatgtcgggcaatcaggtgcgacaatctatcgcttgtatgggaagcccgatgcgccagagttgtttctgaaacatggcaaaggtagcgttgccaatgatgttacagatgagatggtcagactaaactggctgacggaatttatgcctcttccgaccatcaagcattttatccgtactcctgatgatgcatggttactcaccactgcgatccccggaaaaacagcattccaggtattagaagaatatcctgattcaggtgaaaatattgttgatgcgctggcagtgttcctgcgccggttgcattcgattcctgtttgtaattgtccttttaacagcgatcgcgtatttcgtctcgctcaggcgcaatcacgaatgaataacggtttggttgatgcgagtgattttgatgacgagcgtaatggctggcctgttgaacaagtctggaaagaaatgcataaacttttgccattctcaccggattcagtcgtcactcatggtgatttctcacttgataaccttatttttgacgaggggaaattaataggttgtattgatgttggacgagtcggaatcgcagaccgataccaggatcttgccatcctatggaactgcctcggtgagttttctccttcattacagaaacggctttttcaaaaatatggtattgataatcctgatatgaataaattgcagtttcatttgatgctcgatgagtttttctaatcagaattggttaattggttgtaacactggcagagcattacgctgacttgacgggacggcgcaagctcatgaccaaaatcccttaacgtgagttacgcgtgaagatcctttttgataatctcatgaccaaaatcccttaacgtgagttttcgttccactgagcgtcagaccccgtagaaaagatcaaaggatcttcttgagatcctttttttctgcgcgtaatctgctgcttgcaaacaaaaaaaccaccgctaccagcggtggtttgtttgccggatcaagagctaccaactctttttccgaaggtaactggcttcagcagagcgcagataccaaatactgttcttctagtgtagccgtagttaggccaccacttcaagaactctgtagcaccgcctacatacctcgctctgctaatcctgttaccagtggctgctgccagtggcgataagtcgtgtcttaccgggttggactcaagacgatagttaccggataaggcgcagcggtcgggctgaacggggggttcgtgcacacagcccagcttggagcgaacgacctacaccgaactgagatacctacagcgtgagctatgagaaagcgccacgcttcccgaagggagaaaggcggacaggtatccggtaagcggcagggtcggaacaggagagcgcacgagggagcttccagggggaaacgcctggtatctttatagtcctgtcgggtttcgccacctctgacttgagcgtcgatttttgtgatgctcgtcaggggggcggagcctatggaaaaacgccagcaacgcggcctttttacggttcctggccttttgctggccttttgctcacatgt

SEQ ID NO: 30 - DNA, 20 bp, synthetic construct
  source 1..20: mol_type = other DNA
accttcctccatcctccctc

SEQ ID NO: 31 - DNA, 20 bp, synthetic construct
  source 1..20: mol_type = other DNA
tcctgctctgcgaattggtt

SEQ ID NO: 32 - DNA, 20 bp, synthetic construct
  source 1..20: mol_type = other DNA
tccagaaccgccgaatgaaa

SEQ ID NO: 33 - DNA, 20 bp, synthetic construct
  source 1..20: mol_type = other DNA
ccatcagctcctcttccgtc

SEQ ID NO: 34 - DNA, 20 bp, synthetic construct
  source 1..20: mol_type = other DNA
tcctcctgctcaacaacgac

SEQ ID NO: 35 - DNA, 20 bp, synthetic construct
  source 1..20: mol_type = other DNA
cggtccaaggccagaaagat

SEQ ID NO: 36 - DNA, 6209 bp, synthetic construct
  source 1..6209: mol_type = other DNA
cgccatgttgacattgattattgactagttattaatagtaatcaattacggggtcattagttcatagcccatatatggagttccgcgttacataacttacggtaaatggcccgcctggctgaccgcccaacgacccccgcccattgacgtcaataatgacgtatgttcccatagtaacgccaatagggactttccattgacgtcaatgggtggagtatttacggtaaactgcccacttggcagtacatcaagtgtatcatatgccaagtacgccccctattgacgtcaatgacggtaaatggcccgcctggcattatgcccagtacatgaccttatgggactttcctacttggcagtacatctacgtattagtcatcgctattaccatggtgatgcggttttggcagtacatcaatgggcgtggatagcggtttgactcacggggatttccaagtctccaccccattgacgtcaatgggagtttgttttggcaccaaaatcaacgggactttccaaaatgtcgtaacaactccgccccattgacgcaaatgggcggtaggcgtgtacggtgggaggtctatataagcagagctcgtttagtgaaccgtcagatcgcctggagacgccatccacgctgttttgacctccatagaagacaccgggaccgatccagcctcccctcgaagcttacatgtggtaccatggcagcaaggcccaagctccactatcccaacggaagaggccggatggagtccgtgagatgggttttagctgccgccggagtcgagtttgatgaagaatttctggaaacaaaagaacagttgtacaagttgcaggatggtaaccacctgctgttccaacaagtgcccatggttgaaattgacgggatgaagttggtacagacccgaagcattctccactacatagcagacaagcacaatctctttggcaagaacctcaaggagagaaccctgattgacatgtacgtggaggggacactggatctgctggaactgcttatcatgcatcctttcttaaaaccagatgatcagcaaaaggaagtggttaacatggcccagaaggctataattagatactttcctgtgtttgaaaagattttaaggggtcacggacaaagctttcttgttggtaatcagctgagccttgcagatgtgattttactccaaaccattttagctctagaagagaaaattcctaatatcctgtctgcatttcctttcctccaggaatacacagtgaaactaagtaatatccctacaattaagagattccttgaacctggcagcaagaagaagcctccccctgatgaaatttatgtgagaaccgtctacaacatctttaggccataagcggccgctctagaggatccaagcttatcgataccgtcgacctcgagggcccagatctaattcaccccaccagtgcaggctgcctatcagaaagtggtggctggtgtggctaatgccctggcccacaagtatcactaagctcgctttcttgctgtccaatttctattaaaggttcctttgttccctaagtccaactactaaactgggggatattatgaagggccttgagcatctggattctgcctaataaaaaacatttattttcattgcaatgatgtatttaaattatttctgaatattttactaaaaagggaatgtgggaggtcagtgcatttaaaacataaagaaatgaagagctagttcaaaccttgggaaaatacactatatcttaaactccatgaaagaaggtgaggctgcaaacagctaatgcacattggcaacagcccctgatgcctatgccttattcatccctcagaaaaggattcaagtagaggcttgatttggaggttaaagttttgctatgctgtattttacattacttattgttttagctgtcctcatgaatgtcttttcactacccatttgcttatcctgcatctctcagccttgactccactcagttctcttgcttagagataccacctttcccctgaagtgttccttccatgttttacggcgagatggtttctcctcgcctggccactcagccttagttgtctctgttgtcttatagaggtctacttgaagaaggaaaaacagggggcatggtttgactgtcctgtgagcccttcttccctgcctcccccactcacagtgacccggaatccctcgacatctagagcatggctacgtagataagtagcatggcgggttaatcattaactacaaggaacccctagtgatggagttggccactccctctctgcgcgctcgctcgctcactgaggccgggcgaccaaaggtcgcccgacgcccgggctttgcccgggcggcctcagtgagcgagcgagcgcgcagctggcgtaatagcgaagaggcccgcaccgatcgcccttcccaacagttgcgcagcctgaatggcgaatggcgattccgttgcaatggctggcggtaatattgttctggatattaccagcaaggccgatagtttgagttcttctactcaggcaagtgatgttattactaatcaaagaagtattgcgacaacggttaatttgcgtgatggacagactcttttactcggtggcctcactgattataaaaacacttctcaggattctggcgtaccgttcctgtctaaaatccctttaatcggcctcctgtttagctcccgctctgattctaacgaggaaagcacgttatacgtgctcgtcaaagcaaccatagtacgcgccctgtagcggcgcattaagcgcggcgggtgtggtggttacgcgcagcgtgaccgctacacttgccagcgccctagcgcccgctcctttcgctttcttcccttcctttctcgccacgttcgccggctttccccgtcaagctctaaatcgggggctccctttagggttccgatttagtgctttacggcacctcgaccccaaaaaacttgattagggtgatggttcacgtagtgggccatcgccctgatagacggtttttcgccctttgacgttggagtccacgttctttaatagtggactcttgttccaaactggaacaacactcaaccctatctcggtctattcttttgatttataagggattttgccgatttcggcctattggttaaaaaatgagctgatttaacaaaaatttaacgcgaattttaacaaaatattaacgcttacaatttaaatatttgcttatacaatcttcctgtttttggggcttttctgattatcaaccggggtacatatgattgacatgctagttttacgattaccgttcatcgattctcttgtttgctccagactctcaggcaatgacctgatagcctttgtagagacctctcaaaaatagctaccctctccggcatgaatttatcagctagaacggttgaatatcatattgatggtgatttgactgtctccggcctttctcacccgtttgaatctttacctacacattactcaggcattgcatttaaaatatatgagggttctaaaaatttttatccttgcgttgaaataaaggcttctcccgcaaaagtattacagggtcataatgtttttggtacaaccgatttagctttatgctctgaggctttattgcttaattttgctaattctttgccttgcctgtatgatttattggatgttggaatcgcctgatgcggtattttctccttacgcatctgtgcggtatttcacaccgcatatggtgcactctcagtacaatctgctctgatgccgcatagttaagccagccccgacacccgccaacacccgctgacgcgccctgacgggcttgtctgctcccggcatccgcttacagacaagctgtgaccgtctccgggagctgcatgtgtcagaggttttcaccgtcatcaccgaaacgcgcgagacgaaagggcctcgtgatacgcctatttttataggttaatgtcatgataataatggtttcttagacgtcaggtggcacttttcggggaaatgtgcgcggaacccctatttgtttatttttctaaatacattcaaatatgtatccgctcatgagacaataaccctgataaatgcttcaataatattgaaaaaggaagagtatgattgaacaagatggattgcacgcaggttctccggccgcttgggtggagaggctattcggctatgactgggcacaacagacaatcggctgctctgatgccgccgtgttccggctgtcagcgcaggggcgcccggttctttttgtcaagaccgacctgtccggtgccctgaatgaactgcaagacgaggcagcgcggctatcgtggctggccacgacgggcgttccttgcgcagctgtgctcgacgttgtcactgaagcgggaagggactggctgctattgggcgaagtgccggggcaggatctcctgtcatctcaccttgctcctgccgagaaagtatccatcatggctgatgcaatgcggcggctgcatacgcttgatccggctacctgcccattcgaccaccaagcgaaacatcgcatcgagcgagcacgtactcggatggaagccggtcttgtcgatcaggatgatctggacgaagagcatcaggggctcgcgccagccgaactgttcgccaggctcaaggcgagcatgcccgacggcgaggatctcgtcgtgacccatggcgatgcctgcttgccgaatatcatggtggaaaatggccgcttttctggattcatcgactgtggccggctgggtgtggcggaccgctatcaggacatagcgttggctacccgtgatattgctgaagagcttggcggcgaatgggctgaccgcttcctcgtgctttacggtatcgccgctcccgattcgcagcgcatcgccttctatcgccttcttgacgagttcttctgactgtcagaccaagtttactcatatatactttagattgatttaaaacttcatttttaatttaaaaggatctaggtgaagatcctttttgataatctcatgaccaaaatcccttaacgtgagttttcgttccactgagcgtcagaccccgtagaaaagatcaaaggatcttcttgagatcctttttttctgcgcgtaatctgctgcttgcaaacaaaaaaaccaccgctaccagcggtggtttgtttgccggatcaagagctaccaactctttttccgaaggtaactggcttcagcagagcgcagataccaaatactgttcttctagtgtagccgtagttaggccaccacttcaagaactctgtagcaccgcctacatacctcgctctgctaatcctgttaccagtggctgctgccagtggcgataagtcgtgtcttaccgggttggactcaagacgatagttaccggataaggcgcagcggtcgggctgaacggggggttcgtgcacacagcccagcttggagcgaacgacctacaccgaactgagatacctacagcgtgagctatgagaaagcgccacgcttcccgaagggagaaaggcggacaggtatccggtaagcggcagggtcggaacaggagagcgcacgagggagcttccagggggaaacgcctggtatctttatagtcctgtcgggtttcgccacctctgacttgagcgtcgatttttgtgatgctcgtcaggggggcggagcctatggaaaaacgccagcaacgcggcctttttacggttcctggccttttgctggccttttgctcacatgttctttcctgcgttatcccctgattctgtggataaccgtattaccgcctttgagtgagctgataccgctcgccgcagccgaacgaccgagcgcagcgagtcagtgagcgaggaagcggaagagcgcccaatacgcaaaccgcctctccccgcgcgttggccgattcattaatgcagctgcgcgctcgctcgctcactgaggccgcccgggcaaagcccgggcgtcgggcgacctttggtcgcccggcctcagtgagcgagcgagcgcgcagagagggagtggccaactccatcactaggggttccttgtagttaatgattaacccgccatgctacttatctacgtagccatgctctagcggcctcggcctctgcataaataaaaaaaattagtcagccatgagcttggcccattgcatacgttgtatccatatcataatatgtacatttatattggctcatgtccaacattac

SEQ ID NO: 37 - DNA, 589 bp, synthetic construct
  source 1..589: mol_type = other DNA
tagttattaatagtaatcaattacggggtcattagttcatagcccatatatggagttccgcgttacataacttacggtaaatggcccgcctggctgaccgcccaacgacccccgcccattgacgtcaataatgacgtatgttcccatagtaacgccaatagggactttccattgacgtcaatgggtggagtatttacggtaaactgcccacttggcagtacatcaagtgtatcatatgccaagtacgccccctattgacgtcaatgacggtaaatggcccgcctggcattatgcccagtacatgaccttatgggactttcctacttggcagtacatctacgtattagtcatcgctattaccatggtgatgcggttttggcagtacatcaatgggcgtggatagcggtttgactcacggggatttccaagtctccaccccattgacgtcaatgggagtttgttttggcaccaaaatcaacgggactttccaaaatgtcgtaacaactccgccccattgacgcaaatgggcggtaggcgtgtacggtgggaggtctatataagcagagctggtttagtgaaccgtcagatc

SEQ ID NO: 38 - DNA, 66 bp, synthetic construct
  source 1..66: mol_type = other DNA
ggtagcggtgccactaacttctccctgttgaaacaagcaggggatgtcgaagagaatcctggtcca

SEQ ID NO: 39 - DNA, 63 bp, synthetic construct
  source 1..63: mol_type = other DNA
ggcagtggagagggcagaggaagtctgctaacatgcggtgacgtcgaggagaatcctggccca